European Patent Application EP 4 534 667 A1, published April 9, 2025. Title: MODIFIED PROMOTER, EXPRESSION VECTOR, MICROORGANISM, METHOD FOR PRODUCING SUBSTANCE, MODIFIED CYANOBACTERIUM, AND METHOD FOR PREPARING MODIFIED PROMOTER. Applicant: Panasonic Intellectual Property Management Co., Ltd. Application EP. The sequence listing filed with the application follows.

SEQUENCE LISTING (2 sequences)

SEQ ID NO: 1 - DNA, 348 bp, Synechocystis sp.
  source 1..348: mol_type = genomic DNA
gttcagacaaatgctccatcattacgccgggaactatggccggcctaaaaactggccctgcccctagccatcaccaaaatagcaactataatctgttattaaccatcaacatcatcgttccgtgagcagaagctgtaggcggtttttctttaccaacactgattgtggtcctggctccctgagctagcccgcaaaacagaccaatggccttgcttagcctagcatctaccatgaatctaaagaaaattgtcaacttctcccactctttcgaaaaaaacgtgtacaatgtgttactgagtataggacttggttcccgtagtcattattaggtgtgaggaaaagctaaaa

SEQ ID NO: 2 - DNA, 41 bp, Synechocystis sp.
  source 1..41: mol_type = genomic DNA
ttctcccactctttcgaaaaaaacgtgtacaatgtgttact